European Patent Application EP 4 265 640 A2, published October 25, 2023. Title: Polypeptide specific to Mucin1 and use thereof. Applicant: LG CHEM, LTD. The sequence listing filed with the application follows.

SEQUENCE LISTING (115 sequences)

SEQ ID NO: 1 - protein, 8 aa, Artificial Sequence
  2445_1F09 HCDR1
GFTVSSNY

SEQ ID NO: 2 - protein, 7 aa, Artificial Sequence
  2445_1F09 HCDR2
IYSGGST

SEQ ID NO: 3 - protein, 10 aa, Artificial Sequence
  2445_1F09 HCDR3
DRGWNHGMDV

SEQ ID NO: 4 - protein, 8 aa, Artificial Sequence
  2445_1F09 LCDR1
SSEVGSRY

SEQ ID NO: 5 - protein, 3 aa, Artificial Sequence
  2445_1F09 LCDR2
KND

SEQ ID NO: 6 - protein, 11 aa, Artificial Sequence
  2445_1F09 LCDR3
AAWDDSLNGYV

SEQ ID NO: 7 - protein, 118 aa, Artificial Sequence
  2445_1F09 VH
EVQLLETGGGLIQPGGSLRLSCAASGFTVSSNYMSWVRQAPGKGLEWVSVIYSGGSTYYADSVKGRFTISRDNSKNTLYLQMNSLRAEDTAVYYCARDRGWNHGMDVWGQGTLVTVSS

SEQ ID NO: 8 - protein, 110 aa, Artificial Sequence
  2445_1F09 VL
QSGLTQPPSASGTPGQRVTISCSGGSSEVGSRYVSWYQQLPGTAPRLLIYKNDRRPSGVPDRFSGSKSGSSASLAISGLRSEDEADYYCAAWDDSLNGYVFGTGTKLTVL

SEQ ID NO: 9 - protein, 243 aa, Artificial Sequence
  2445_1F09 scFv
EVQLLETGGGLIQPGGSLRLSCAASGFTVSSNYMSWVRQAPGKGLEWVSVIYSGGSTYYADSVKGRFTISRDNSKNTLYLQMNSLRAEDTAVYYCARDRGWNHGMDVWGQGTLVTVSSGGGGSGGGGSGGGASQSGLTQPPSASGTPGQRVTISCSGGSSEVGSRYVSWYQQLPGTAPRLLIYKNDRRPSGVPDRFSGSKSGSSASLAISGLRSEDEADYYCAAWDDSLNGYVFGTGTKLTVL

SEQ ID NO: 10 - DNA, 729 bp, Artificial Sequence
  2445_1F09 scFv
gaggtgcagctgttggagactggaggaggcttgatccagcctggggggtccctgagactctcctgtgcagcctctgggttcaccgtcagtagcaactacatgagctgggtccgccaggctccagggaaggggctggagtgggtctcagttatttatagcggtggtagcacatattacgcagactccgtgaagggccgattcaccatctccagagacaattccaagaacacgctgtatcttcaaatgaacagcctgagagccgaggacacggccgtgtattactgtgcgagagatcgcggctggaaccacggtatggacgtctggggccagggaaccctggtcaccgtctcgagtggtggaggcggttcaggcggaggtggctctggcggtggcgctagccagtctgggctgactcagccaccctcagcgtctgggacccccgggcagagggtcaccatctcttgttctgggggcagctcagaagtcggaagtagatatgtgtcctggtaccagcaactcccaggaacggcccccagactcctcatctataagaatgatcggcggccctcaggggtccctgaccgattctctggctccaagtctggctcctcagcctccctggccatcagtgggctccggtccgaggatgaggctgattattactgtgcagcatgggatgacagcctgaatggttatgtcttcggaactgggaccaagctgaccgtccta

SEQ ID NO: 11 - protein, 8 aa, Artificial Sequence
  2447_2H08 HCDR1
GYTFTNYG

SEQ ID NO: 12 - protein, 8 aa, Artificial Sequence
  2447_2H08 HCDR2
ISAYNGNT

SEQ ID NO: 13 - protein, 16 aa, Artificial Sequence
  2447_2H08 HCDR3
DPHILTGYYRGGWFDP

SEQ ID NO: 14 - protein, 6 aa, Artificial Sequence
  2447_2H08 LCDR1
SLRTSY

SEQ ID NO: 15 - protein, 3 aa, Artificial Sequence
  2447_2H08 LCDR2
GKT

SEQ ID NO: 16 - protein, 13 aa, Artificial Sequence
  2447_2H08 LCDR3
HSRDSNDNYLEVV

SEQ ID NO: 17 - protein, 125 aa, Artificial Sequence
  2447_2H08 VH
EVQLVQSGAEVKKPGASVKVSCKASGYTFTNYGISWVRQAPGQGLEWMGWISAYNGNTNYAQKLQGRVTMTTDTSTSTAYMELRSLRSDDTAVYYCARDPHILTGYYRGGWFDPWGQGTTVTVSS

SEQ ID NO: 18 - protein, 110 aa, Artificial Sequence
  2447_2H08 VL
SYELTQDPAVSVALGQTVTITCQGDSLRTSYAGWLQQKPGQAPVLVLYGKTSRPSGIPDRFSGSTSGNTASLTITGAQAEDEAEYFCHSRDSNDNYLEVVFGGGTKLTVL

SEQ ID NO: 19 - protein, 250 aa, Artificial Sequence
  2447_2H08 scFv
EVQLVQSGAEVKKPGASVKVSCKASGYTFTNYGISWVRQAPGQGLEWMGWISAYNGNTNYAQKLQGRVTMTTDTSTSTAYMELRSLRSDDTAVYYCARDPHILTGYYRGGWFDPWGQGTTVTVSSGGGGSGGGGSGGGASSYELTQDPAVSVALGQTVTITCQGDSLRTSYAGWLQQKPGQAPVLVLYGKTSRPSGIPDRFSGSTSGNTASLTITGAQAEDEAEYFCHSRDSNDNYLEVVFGGGTKLTVL

SEQ ID NO: 20 - DNA, 750 bp, Artificial Sequence
  2447_2H08 scFv
gaagtgcagctggtgcagtctggagctgaggtgaagaagcctggggcctcagtgaaggtctcctgcaaggcttctggttacacctttaccaactacggtatcagctgggtgcgacaggcccctggacaagggcttgagtggatgggatggatcagcgcttacaatggtaacacaaactatgcacagaagctccagggcagagtcaccatgaccacagacacatccacgagcacagcctacatggagctgaggagcctgagatctgacgacacggccgtgtattactgtgcgagagatccgcatattttgactggttattataggggagggtggttcgacccctgggggcaagggaccacggtcaccgtctcgagtggtggaggcggttcaggcggaggtggctctggcggtggcgctagctcctatgagctgactcaggaccctgctgtgtctgtggccttgggtcagacagtcaccatcacgtgccaaggagacagcctcagaacctcttatgcaggctggctccagcagaagccaggacaggcccctgtactcgtcctctatggtaaaaccagccggccctcagggatcccagaccgattctctggctccacctcaggaaacacagcttccttgaccatcactggggctcaggcggaggatgaggctgagtatttctgtcactcccgggacagcaatgataactatctagaggtggttttcggcggagggaccaagctgaccgtccta

SEQ ID NO: 21 - protein, 8 aa, Artificial Sequence
  2447_3A01 HCDR1
GFTFDDYA

SEQ ID NO: 22 - protein, 8 aa, Artificial Sequence
  2447_3A01 HCDR2
ISWNSGSI

SEQ ID NO: 23 - protein, 13 aa, Artificial Sequence
  2447_3A01 HCDR3
DISSGWYPGTFDY

SEQ ID NO: 24 - protein, 6 aa, Artificial Sequence
  2447_3A01 LCDR1
SLRSYY

SEQ ID NO: 25 - protein, 3 aa, Artificial Sequence
  2447_3A01 LCDR2
GKN

SEQ ID NO: 26 - protein, 10 aa, Artificial Sequence
  2447_3A01 LCDR3
SSRDSSDDVV

SEQ ID NO: 27 - protein, 122 aa, Artificial Sequence
  2447_3A01 VH
EVQLLESGGGLVQPGGSLRLSCAASGFTFDDYAMHWVRQAPGKGLEWVSGISWNSGSIVYADFVKGRFTISRDNAKNSLYLQMNSLRAEDTALYYCAKDISSGWYPGTFDYWGQGTLVTVSS

SEQ ID NO: 28 - protein, 107 aa, Artificial Sequence
  2447_3A01 VL
SYELTQDPAVSVALGQTVRITCQGDSLRSYYASWYQQKPGQAPVLVIYGKNNRPSGIPDRFSGSSSGNTASLTVTGAQAEDEADYYCSSRDSSDDVVFGGGTQLTVL

SEQ ID NO: 29 - protein, 244 aa, Artificial Sequence
  2447_3A01 scFv
EVQLLESGGGLVQPGGSLRLSCAASGFTFDDYAMHWVRQAPGKGLEWVSGISWNSGSIVYADFVKGRFTISRDNAKNSLYLQMNSLRAEDTALYYCAKDISSGWYPGTFDYWGQGTLVTVSSGGGGSGGGGSGGGASSYELTQDPAVSVALGQTVRITCQGDSLRSYYASWYQQKPGQAPVLVIYGKNNRPSGIPDRFSGSSSGNTASLTVTGAQAEDEADYYCSSRDSSDDVVFGGGTQLTVL

SEQ ID NO: 30 - DNA, 732 bp, Artificial Sequence
  2447_3A01 scFv
gaggtgcagctgttggagtctgggggaggcttggtacagcctggggggtccctgagactctcctgtgcagcctctggattcacctttgatgattatgccatgcactgggtccggcaagctccagggaagggcctggagtgggtctcaggtattagttggaatagtggtagcatagtctatgcggactttgtgaagggccgattcaccatctccagagacaacgccaagaactccctgtatctgcaaatgaacagtctgagagctgaggacacggccttgtattactgtgcaaaagatatttcaagtggctggtacccagggacctttgactactggggccagggaaccctggtcaccgtctcgagtggtggaggcggttcaggcggaggtggctctggcggtggcgctagctcctatgagctgactcaggaccctgctgtgtctgtggccttgggacagacagtcaggatcacatgccaaggagacagcctcagaagctattatgcaagctggtaccagcagaagccaggacaggcccctgtacttgtcatctatggtaaaaacaaccggccctcagggatcccagaccgattctctggctccagctcaggaaacacagcttccttgaccgtcactggggctcaggcggaagacgaggctgactattactgtagctcccgggacagcagtgatgatgtggtattcggcggagggacccagctcaccgtccta

SEQ ID NO: 31 - protein, 8 aa, Artificial Sequence
  2447_3A08 HCDR1
GYTFTSYG

SEQ ID NO: 32 - protein, 8 aa, Artificial Sequence
  2447_3A08 HCDR2
ISAYNGNT

SEQ ID NO: 33 - protein, 14 aa, Artificial Sequence
  2447_3A08 HCDR3
DRATIFGVVTPFDY

SEQ ID NO: 34 - protein, 6 aa, Artificial Sequence
  2447_3A08 LCDR1
SIRSYS

SEQ ID NO: 35 - protein, 3 aa, Artificial Sequence
  2447_3A08 LCDR2
GKN

SEQ ID NO: 36 - protein, 11 aa, Artificial Sequence
  2447_3A08 LCDR3
NSRDSSGNRVV

SEQ ID NO: 37 - protein, 123 aa, Artificial Sequence
  2447_3A08 VH
EVQLVQSGAEVKKPGASVKVSCKASGYTFTSYGISWVRQAPGQGLEWMGWISAYNGNTNYAQKLQGRVTMTTDTSTSTAYMELRSLRSDDTAVYYCARDRATIFGVVTPFDYWGQGTLVTVSS

SEQ ID NO: 38 - protein, 108 aa, Artificial Sequence
  2447_3A08 VL
SYELTQDPAVSVALGQTVRITCQGDSIRSYSASWYQQKPGQAPRLVIYGKNNRPSGIPDRVSGSTSGNTASLTVTGAQAEDEADYYCNSRDSSGNRVVFGGGTQLTVL

SEQ ID NO: 39 - protein, 246 aa, Artificial Sequence
  2447_3A08 scFv
EVQLVQSGAEVKKPGASVKVSCKASGYTFTSYGISWVRQAPGQGLEWMGWISAYNGNTNYAQKLQGRVTMTTDTSTSTAYMELRSLRSDDTAVYYCARDRATIFGVVTPFDYWGQGTLVTVSSGGGGSGGGGSGGGASSYELTQDPAVSVALGQTVRITCQGDSIRSYSASWYQQKPGQAPRLVIYGKNNRPSGIPDRVSGSTSGNTASLTVTGAQAEDEADYYCNSRDSSGNRVVFGGGTQLTVL

SEQ ID NO: 40 - DNA, 738 bp, Artificial Sequence
  2447_3A08 scFv
gaagtgcagctggtgcagtctggagctgaggtgaagaagcctggggcctcagtgaaggtctcctgcaaggcttctggttacacctttaccagctacggtatcagctgggtgcgacaggcccctggacaagggcttgagtggatgggatggatcagcgcttacaatggtaacacaaactatgcacagaagctccagggcagagtcaccatgaccacagacacatccacgagcacagcctacatggagctgaggagcctgagatctgacgacacggccgtgtattactgtgcgagagatcgggctacgatttttggagtggttaccccctttgactactggggccaaggaaccctggtcaccgtctcgagtggtggaggcggttcaggcggaggtggctctggcggtggcgctagctcctatgagctgactcaggaccccgctgtgtctgtggccttgggacagacagtcaggatcacatgccagggagacagtattagaagttattctgccagctggtaccagcagaagccagggcaggcccctcgccttgttatctatggtaaaaacaaccggccctcagggatcccagaccgagtctctggctccacttcaggaaatacagcttccttgaccgtcactggggctcaggcggaagatgaggctgactattactgtaactcccgggacagcagtggtaaccgtgtggtattcggcggagggacccagctcaccgtccta

SEQ ID NO: 41 - protein, 8 aa, Artificial Sequence
  2447_3A09 HCDR1
GFTFDDYA

SEQ ID NO: 42 - protein, 8 aa, Artificial Sequence
  2447_3A09 HCDR2
ISWNSGSI

SEQ ID NO: 43 - protein, 13 aa, Artificial Sequence
  2447_3A09 HCDR3
DVSSGWYWYAFDI

SEQ ID NO: 44 - protein, 6 aa, Artificial Sequence
  2447_3A09 LCDR1
SLRSYY

SEQ ID NO: 45 - protein, 3 aa, Artificial Sequence
  2447_3A09 LCDR2
GKN

SEQ ID NO: 46 - protein, 10 aa, Artificial Sequence
  2447_3A09 LCDR3
NSRDSGGSVV

SEQ ID NO: 47 - protein, 122 aa, Artificial Sequence
  2447_3A09 VH
EVQLLESGGGLVQPGRSLRLSCAATGFTFDDYAMHWVRQAPGKGLEWVSGISWNSGSIGYADSVKGRFTISRDNAKNSLYLQMNSLRAEDTASYYCAKDVSSGWYWYAFDIWGQGTLVTVSS

SEQ ID NO: 48 - protein, 107 aa, Artificial Sequence
  2447_3A09 VL
SYELTQDPAVSVALGQTVRITCQGDSLRSYYASWYQQKPGQAPVLVIYGKNNRPSGIPGRFSGSSSGNTASLTVTGAQAEDEADYYCNSRDSGGSVVFGGGTKLTVL

SEQ ID NO: 49 - protein, 244 aa, Artificial Sequence
  2447_3A09 scFv
EVQLLESGGGLVQPGRSLRLSCAATGFTFDDYAMHWVRQAPGKGLEWVSGISWNSGSIGYADSVKGRFTISRDNAKNSLYLQMNSLRAEDTASYYCAKDVSSGWYWYAFDIWGQGTLVTVSSGGGGSGGGGSGGGASSYELTQDPAVSVALGQTVRITCQGDSLRSYYASWYQQKPGQAPVLVIYGKNNRPSGIPGRFSGSSSGNTASLTVTGAQAEDEADYYCNSRDSGGSVVFGGGTKLTVL

SEQ ID NO: 50 - DNA, 732 bp, Artificial Sequence
  2447_3A09 scFv
gaggtgcagctgttggagtctgggggaggcttggtacagcctggcaggtccctgagactctcctgtgcagccactggattcacctttgatgattatgccatgcactgggtccggcaagctccagggaagggcctggagtgggtctcaggtattagttggaatagtggtagcataggctatgcggactctgtgaagggccgattcaccatctccagagacaacgccaagaactccctgtatctgcaaatgaacagtctgagagctgaggacacggcctcgtattactgtgcaaaagatgttagcagtggctggtactggtatgcttttgatatctggggccaaggaaccctggtcaccgtctcgagtggtggaggcggttcaggcggaggtggctctggcggtggcgctagctcctatgagctgactcaggaccctgctgtgtctgtggccttgggacagacagtcaggatcacatgccaaggagacagcctcagaagctattatgcaagctggtaccagcagaagccaggacaggcccctgtacttgtcatctatggtaaaaacaaccggccctcagggatcccaggccgattctctggctccagctcaggaaacacagcttccttgaccgtcactggggctcaggcggaagatgaggctgactattactgtaattcccgggacagcggtggttctgtggttttcggcggagggaccaagctgaccgtccta

SEQ ID NO: 51 - protein, 8 aa, Artificial Sequence
  2447_3A12 HCDR1
GYTFTSYG

SEQ ID NO: 52 - protein, 8 aa, Artificial Sequence
  2447_3A12 HCDR2
ISAYNGNT

SEQ ID NO: 53 - protein, 16 aa, Artificial Sequence
  2447_3A12 HCDR3
DPHILTGYYRGGWFDP

SEQ ID NO: 54 - protein, 6 aa, Artificial Sequence
  2447_3A12 LCDR1
SLRSYY

SEQ ID NO: 55 - protein, 3 aa, Artificial Sequence
  2447_3A12 LCDR2
GKN

SEQ ID NO: 56 - protein, 11 aa, Artificial Sequence
  2447_3A12 LCDR3
NSRDSSGNHRV

SEQ ID NO: 57 - protein, 125 aa, Artificial Sequence
  2447_3A12 VH
EVQLVQSGAEVKKPGASVKVSCKASGYTFTSYGISWVRQAPGQGLEWMGWISAYNGNTNYAQKLRGRVTMTTDTSTSTAYMELRSLRSDDTAVYYCARDPHILTGYYRGGWFDPWGQGTLVTVSS

SEQ ID NO: 58 - protein, 108 aa, Artificial Sequence
  2447_3A12 VL
SYELTQDPAVSVVLGQTVRITCQGDSLRSYYASWYQQKPGQAPVLVIYGKNNRPSGIPDRFSGSSSGNTASLTITGAQAEDEADYYCNSRDSSGNHRVFGGGTKLTVL

SEQ ID NO: 59 - protein, 248 aa, Artificial Sequence
  2447_3A12 scFv
EVQLVQSGAEVKKPGASVKVSCKASGYTFTSYGISWVRQAPGQGLEWMGWISAYNGNTNYAQKLRGRVTMTTDTSTSTAYMELRSLRSDDTAVYYCARDPHILTGYYRGGWFDPWGQGTLVTVSSGGGGSGGGGSGGGASSYELTQDPAVSVVLGQTVRITCQGDSLRSYYASWYQQKPGQAPVLVIYGKNNRPSGIPDRFSGSSSGNTASLTITGAQAEDEADYYCNSRDSSGNHRVFGGGTKLTVL

SEQ ID NO: 60 - DNA, 744 bp, Artificial Sequence
  2447_3A12 scFv
gaagtgcagctggtgcagtctggagctgaggtgaagaagcctggggcctcagtgaaggtctcctgcaaggcttctggttacacctttaccagctatggtatcagctgggtgcgacaggcccctggacaagggcttgagtggatgggatggatcagcgcttacaatggtaacacaaactatgcacagaagctccggggcagagtcaccatgaccacagacacatccacgagcacagcctacatggagctgaggagcctgagatctgacgacacggccgtgtattactgtgcgagagatccgcatattttgactggttattataggggagggtggttcgacccctggggccagggcaccctggtcaccgtctcgagtggtggaggcggttcaggcggaggtggctctggcggtggcgctagctcctatgagctgactcaggaccctgctgtgtctgtggtcttgggacagacagtcaggatcacatgccaaggagacagcctcagaagctattatgcaagctggtaccagcagaagccaggacaggcccctgtacttgtcatctatggtaaaaacaaccggccctcagggatcccagaccgattctctggctccagctcaggaaacacagcttccttgaccatcactggggctcaggcggaagatgaggctgactattactgtaactcccgggacagcagtggtaaccatcgtgtattcggcggagggaccaagctgaccgtccta

SEQ ID NO: 61 - protein, 8 aa, Artificial Sequence
  2447_3B07 HCDR1
GFTFDDYA

SEQ ID NO: 62 - protein, 8 aa, Artificial Sequence
  2447_3B07 HCDR2
TSWDGGST

SEQ ID NO: 63 - protein, 10 aa, Artificial Sequence
  2447_3B07 HCDR3
DHSSGWYNGG

SEQ ID NO: 64 - protein, 6 aa, Artificial Sequence
  2447_3B07 LCDR1
SLRSYY

SEQ ID NO: 65 - protein, 3 aa, Artificial Sequence
  2447_3B07 LCDR2
GKN

SEQ ID NO: 66 - protein, 11 aa, Artificial Sequence
  2447_3B07 LCDR3
NSRDSSGNHVV

SEQ ID NO: 67 - protein, 122 aa, Artificial Sequence
  2447_3B07 VH
QVQLVESGGVVVQPGGSLRLSCAASGFTFDDYAMHWVRQAPGRGLEWVSLTSWDGGSTYYADSVKGRFTISRDNSKNSLYLQMNSLRAEDTALYYCAKDHSSGWYNGGMDVWGQGTMVTVSS

SEQ ID NO: 68 - protein, 108 aa, Artificial Sequence
  2447_3B07 VL
SYELTQDPAVSVALGQTVRITCQGDSLRSYYASWYQQKPGQAPVLVIYGKNNRPSGIPDRFSGSSSGNTASLTITGAQAEDEADYYCNSRDSSGNHVVFGGGTKLTVL

SEQ ID NO: 69 - protein, 245 aa, Artificial Sequence
  2447_3B07 scFv
QVQLVESGGVVVQPGGSLRLSCAASGFTFDDYAMHWVRQAPGRGLEWVSLTSWDGGSTYYADSVKGRFTISRDNSKNSLYLQMNSLRAEDTALYYCAKDHSSGWYNGGMDVWGQGTMVTVSSGGGGSGGGGSGGGASSYELTQDPAVSVALGQTVRITCQGDSLRSYYASWYQQKPGQAPVLVIYGKNNRPSGIPDRFSGSSSGNTASLTITGAQAEDEADYYCNSRDSSGNHVVFGGGTKLTVL

SEQ ID NO: 70 - DNA, 735 bp, Artificial Sequence
  2447_3B07 scFv
caggtgcagctggtggagtctgggggagtcgtggtacagcctggggggtccctgagactctcctgtgcagcctctggattcacctttgatgattatgccatgcactgggtccgtcaagctccggggaggggtctggagtgggtctctcttactagttgggatggtggtagcacatactatgcagactctgtgaagggtcgattcaccatctccagagacaacagcaaaaactccctgtatctgcaaatgaacagtctgagagctgaggacaccgccttgtattactgtgcaaaagatcatagcagcggctggtacaacgggggtatggacgtctggggccaagggacaatggtcaccgtctcgagtggtggaggcggttcaggcggaggtggctctggcggtggcgctagctcctatgagctgactcaggaccctgctgtgtctgtggccttgggacagacagtcaggatcacatgccaaggagacagcctcagaagctattatgcaagctggtaccagcagaagccaggacaggcccctgtacttgtcatctatggtaaaaacaaccggccctcagggatcccagaccgattctctggctccagctcaggaaacacagcttccttgaccatcactggggctcaggcggaagatgaggctgactattactgtaactcccgggacagcagtggtaaccatgtggtattcggcggagggaccaagctgaccgtccta

SEQ ID NO: 71 - protein, 8 aa, Artificial Sequence
  2447_3C08 HCDR1
GFTFDDYA

SEQ ID NO: 72 - protein, 8 aa, Artificial Sequence
  2447_3C08 HCDR2
ISWNSGSI

SEQ ID NO: 73 - protein, 15 aa, Artificial Sequence
  2447_3C08 HCDR3
DRGSGYEGNYYGMDV

SEQ ID NO: 74 - protein, 6 aa, Artificial Sequence
  2447_3C08 LCDR1
SLRSYY

SEQ ID NO: 75 - protein, 3 aa, Artificial Sequence
  2447_3C08 LCDR2
GKN

SEQ ID NO: 76 - protein, 11 aa, Artificial Sequence
  2447_3C08 LCDR3
NSRDSSGNHYV

SEQ ID NO: 77 - protein, 124 aa, Artificial Sequence
  2447_3C08 VH
EVQLLESGGGLVQPGGSLRLSCAASGFTFDDYAMHWVRQAPGKGLEWVSGISWNSGSIGYADSVKGRFTISRDNAKNSLYLQMNSLRAEDTALYYCAKDRGSGYEGNYYGMDVWGQGTLVTVSS

SEQ ID NO: 78 - protein, 108 aa, Artificial Sequence
  2447_3C08 VL
SYELTQDPAVSVALGQTVRITCQGDSLRSYYASWYQQKPGQAPVLVIYGKNNRPSGIPDRFSGTTSGNTASLTITGAQAEDEADYYCNSRDSSGNHYVFGTGTKVTVL

SEQ ID NO: 79 - protein, 247 aa, Artificial Sequence
  2447_3C08 scFv
EVQLLESGGGLVQPGGSLRLSCAASGFTFDDYAMHWVRQAPGKGLEWVSGISWNSGSIGYADSVKGRFTISRDNAKNSLYLQMNSLRAEDTALYYCAKDRGSGYEGNYYGMDVWGQGTLVTVSSGGGGSGGGGSGGGASSYELTQDPAVSVALGQTVRITCQGDSLRSYYASWYQQKPGQAPVLVIYGKNNRPSGIPDRFSGTTSGNTASLTITGAQAEDEADYYCNSRDSSGNHYVFGTGTKVTVL

SEQ ID NO: 80 - DNA, 741 bp, Artificial Sequence
  2447_3C08 scFv
gaggtgcagctgttggagtctgggggaggcttggtacagcctggggggtccctgagactctcctgtgcagcctctggattcacctttgatgattatgccatgcactgggtccggcaagctccagggaagggcctggagtgggtctcaggtattagttggaatagtggtagcataggctatgcggactctgtgaagggccgattcaccatctccagagacaacgccaagaactccctgtatctgcaaatgaacagtctgagagctgaggacacggccttgtattactgtgcaaaagataggggtagtggctacgaaggaaactactacggtatggacgtctggggccaaggaaccctggtcaccgtctcgagtggtggaggcggttcaggcggaggtggctctggcggtggcgctagctcctatgagctgactcaggaccctgctgtgtctgtggccttgggacagacagtcaggatcacatgccaaggagacagcctcagaagctattatgcaagctggtaccagcagaagccaggacaggcccctgtacttgtcatctatggtaaaaacaaccggccctcagggatcccagaccgattctctggtaccacctcaggaaacacagcctccttgaccatcactggggctcaggcggaagatgaggctgactattactgtaactcccgggacagcagtggtaaccattatgtcttcggaactgggaccaaggtcaccgtccta

SEQ ID NO: 81 - protein, 8 aa, Artificial Sequence
  2447_3H02 HCDR1
GFTFDDYA

SEQ ID NO: 82 - protein, 8 aa, Artificial Sequence
  2447_3H02 HCDR2
ISWDSGSI

SEQ ID NO: 83 - protein, 13 aa, Artificial Sequence
  2447_3H02 HCDR3
DVSSGWYWYAFDI

SEQ ID NO: 84 - protein, 6 aa, Artificial Sequence
  2447_3H02 LCDR1
ILRSYY

SEQ ID NO: 85 - protein, 3 aa, Artificial Sequence
  2447_3H02 LCDR2
GKN

SEQ ID NO: 86 - protein, 11 aa, Artificial Sequence
  2447_3H02 LCDR3
NSRDSSGNRVV

SEQ ID NO: 87 - protein, 122 aa, Artificial Sequence
  2447_3H02 VH
EVQLLESGGGLVQPGRSLRLSCAASGFTFDDYAMHWVRQAPGKGLEWVSGISWDSGSIGYADSVKGRFTISRDNAKNSLYLQMNSLRAEDTALYYCAKDVSSGWYWYAFDIWGQGTLVTVSS

SEQ ID NO: 88 - protein, 108 aa, Artificial Sequence
  2447_3H02 VL
SYELTQDPAVSVALGQTVRITCQGDILRSYYASWYQQKPGQAPVLVIYGKNNRPSGIPDRFSGSSSGNTASLTITGAQAEDEADYYCNSRDSSGNRVVFGGGTKLTVL

SEQ ID NO: 89 - protein, 245 aa, Artificial Sequence
  2447_3H02 scFv
EVQLLESGGGLVQPGRSLRLSCAASGFTFDDYAMHWVRQAPGKGLEWVSGISWDSGSIGYADSVKGRFTISRDNAKNSLYLQMNSLRAEDTALYYCAKDVSSGWYWYAFDIWGQGTLVTVSSGGGGSGGGGSGGGASSYELTQDPAVSVALGQTVRITCQGDILRSYYASWYQQKPGQAPVLVIYGKNNRPSGIPDRFSGSSSGNTASLTITGAQAEDEADYYCNSRDSSGNRVVFGGGTKLTVL

SEQ ID NO: 90 - DNA, 735 bp, Artificial Sequence
  2447_3H02 scFv
gaggtgcagctgttggagtctgggggaggcttggtacagcctggcaggtccctgagactctcctgtgcagcctctggattcacctttgatgattatgccatgcactgggtccggcaagctccagggaagggcctggagtgggtctcaggtattagttgggatagtggtagcataggctatgcggactctgtgaagggccgattcaccatctccagagacaacgccaagaactccctgtatctgcaaatgaacagtctgagagctgaggacacggccttgtattactgtgcaaaagatgttagcagtggctggtactggtatgcttttgatatctggggccagggaaccctggtcaccgtctcgagtggtggaggcggttcaggcggaggtggctctggcggtggcgctagctcctatgagctgactcaggaccctgctgtgtctgtggccttgggacagacagtcaggatcacatgccaaggagacatcctcagaagttattatgcaagttggtaccagcagaagccaggacaggcccctgtacttgtcatttatggtaaaaacaaccggccctcagggatcccagaccgattctctggctccagctcaggaaacacagcttccttgaccatcactggggctcaggcggaagatgaggctgactattactgtaactcccgggacagcagtggtaaccgtgtggtattcggcggagggaccaagctgaccgtccta

SEQ ID NO: 91 - protein, 8 aa, Artificial Sequence
  2447_3H08 HCDR1
GFTFDDYA

SEQ ID NO: 92 - protein, 8 aa, Artificial Sequence
  2447_3H08 HCDR2
ISWNSGSI

SEQ ID NO: 93 - protein, 13 aa, Artificial Sequence
  2447_3H08 HCDR3
DRSSGWYTGSFDY

SEQ ID NO: 94 - protein, 6 aa, Artificial Sequence
  2447_3H08 LCDR1
SLRSYY

SEQ ID NO: 95 - protein, 3 aa, Artificial Sequence
  2447_3H08 LCDR2
GKN

SEQ ID NO: 96 - protein, 11 aa, Artificial Sequence
  2447_3H08 LCDR3
QSRDSSDNRVL

SEQ ID NO: 97 - protein, 122 aa, Artificial Sequence
  2447_3H08 VH
EVQLLESGGGLVQPGRSLRLSCAASGFTFDDYAMHWVRQAPGKGLEWVSGISWNSGSIDYADSVKGRFTISRDNSKNTLYLQMNSLRAEDTAVYYCARDRSSGWYTGSFDYWGQGTLVTVSS

SEQ ID NO: 98 - protein, 108 aa, Artificial Sequence
  2447_3H08 VL
SYELTQDPAVSVALGQTVRITCQGDSLRSYYASWYRQKPGQAPVLVIYGKNNRPSGIPDRFSGSSSGNTASLTIIGAQAEDEADYYCQSRDSSDNRVLFGGGTKVTVL

SEQ ID NO: 99 - protein, 245 aa, Artificial Sequence
  2447_3H08 scFv
EVQLLESGGGLVQPGRSLRLSCAASGFTFDDYAMHWVRQAPGKGLEWVSGISWNSGSIDYADSVKGRFTISRDNSKNTLYLQMNSLRAEDTAVYYCARDRSSGWYTGSFDYWGQGTLVTVSSGGGGSGGGGSGGGASSYELTQDPAVSVALGQTVRITCQGDSLRSYYASWYRQKPGQAPVLVIYGKNNRPSGIPDRFSGSSSGNTASLTIIGAQAEDEADYYCQSRDSSDNRVLFGGGTKVTVL

SEQ ID NO: 100 - DNA, 735 bp, Artificial Sequence
  2447_3H08 scFv
gaggtgcagctgttggagtctgggggaggcttggtacagcctggcaggtccctgagactctcctgtgcagcctctggattcacctttgatgattatgccatgcactgggtccggcaagctccagggaagggcctggagtgggtctcaggtattagttggaatagtggtagcatagactatgcagactccgtgaagggccgattcaccatctccagagacaattccaagaacacgctgtatctgcaaatgaacagcctgagagctgaggacacagctgtgtactactgtgcgagagatcggagtagtggctggtacacggggtcctttgactactggggccagggcaccctggtcaccgtctcgagtggtggaggcggttcaggcggaggtggctctggcggtggcgctagctcctatgagctgactcaggaccctgctgtgtctgtggccttgggacagacagtcaggatcacatgccaaggagacagcctcagaagctattatgcaagctggtaccggcagaagccaggacaggcccctgtacttgtcatctatggtaaaaacaaccggccctcagggatcccagaccgattctctggctccagctcgggaaacacagcttccttgaccatcattggggctcaggcggaagacgaggctgactattactgtcagtcccgggacagcagtgataaccgtgttctattcggcggagggaccaaggtcaccgtccta

SEQ ID NO: 101 - protein, 8 aa, Artificial Sequence
  G03 HCDR1
GYTFTSYW

SEQ ID NO: 102 - protein, 8 aa, Artificial Sequence
  G03 HCDR2
INPGTGYI

SEQ ID NO: 103 - protein, 7 aa, Artificial Sequence
  G03 HCDR3
STAPFDY

SEQ ID NO: 104 - protein, 6 aa, Artificial Sequence
  G03 LCDR1
QDIKSY

SEQ ID NO: 105 - protein, 3 aa, Artificial Sequence
  G03 LCDR2
YAT

SEQ ID NO: 106 - protein, 9 aa, Artificial Sequence
  G03 LCDR3
LQYDESPYT

SEQ ID NO: 107 - protein, 116 aa, Artificial Sequence
  G03 VH
EVQLVQSGAEVKKPGATVKISCKVSGYTFTSYWMHWVQQAPGKGLEWIGYINPGTGYIEYNQKFKDRVTITADKSTDTAYMELSSLRSEDTAVYYCASSTAPFDYWGQGTLVTVSS

SEQ ID NO: 108 - protein, 107 aa, Artificial Sequence
  G03 VL
EIVLTQSPGTLSLSPGERATLSCKASQDIKSYLSWYQQKPGQAPRLLIYYATRLADGIPDRFSGSGSGTDFTLTISRLEPEDFAVYYCLQYDESPYTFGQGTKLEIK

SEQ ID NO: 109 - protein, 238 aa, Artificial Sequence
  G03 scFv
EVQLVQSGAEVKKPGATVKISCKVSGYTFTSYWMHWVQQAPGKGLEWIGYINPGTGYIEYNQKFKDRVTITADKSTDTAYMELSSLRSEDTAVYYCASSTAPFDYWGQGTLVTVSSGGGGSGGGGSGGGASEIVLTQSPGTLSLSPGERATLSCKASQDIKSYLSWYQQKPGQAPRLLIYYATRLADGIPDRFSGSGSGTDFTLTISRLEPEDFAVYYCLQYDESPYTFGQGTKLEIK

SEQ ID NO: 110 - protein, 113 aa, Artificial Sequence
  mucin 1
SFFFLSFHISNLQFNSSLEDPSTDYYQELQRDISEMFLQIYKQGGFLGLSNIKFRPGSVVVQLTLAFREGTINVHDVETQFNQYKTEAASRYNLTISDVSVSDVPFPFSAQSG

SEQ ID NO: 111 - protein, 182 aa, Artificial Sequence
  Synthetic_CD4
TSITAYKSEGESAEFSFPLNLGEESLQGELRWKAEKAPSSQSWITFSLKNQKVSVQKSTSNPKFQLSETLPLTLQIPQVSLQFAGSGNLTLTLDRGILYQEVNLVVMKVTQPDSNTLTCEVMGPTSPKMRLILKQENQEARVSRQEKVIQVQAPEAGVWQCLLSEGEEVKMDSKIQVLSKGL

SEQ ID NO: 112 - DNA, 135 bp, Artificial Sequence
  hinge domain
accacgacgccagcgccgcgaccaccaacaccggcgcccaccatcgcgtcgcagcccctgtccctgcgcccagaggcgtgccggccagcggcggggggcgcagtgcacacgagggggctggacttcgcctgtgat

SEQ ID NO: 113 - DNA, 81 bp, Artificial Sequence
  CD28 transmembrane domain
ttttgggtgctggtggtggttggtggagtcctggcttgctatagcttgctagtaacagtggcctttattattttctgggtg

SEQ ID NO: 114 - DNA, 123 bp, Artificial Sequence
  CD28 costimulatory domain
aggagtaagaggagcaggctcctgcacagtgactacatgaacatgactccccgccgccccgggcccacccgcaagcattaccagccctatgccccaccacgcgacttcgcagcctatcgctcc

SEQ ID NO: 115 - DNA, 336 bp, Artificial Sequence
  CD3 zeta intracellular signaling domain
agagtgaagttcagcaggagcgcagacgcccccgcgtaccagcagggccagaaccagctctataacgagctcaatctaggacgaagagaggagtacgatgttttggacaagagacgtggccgggaccctgagatggggggaaagccgagaaggaagaaccctcaggaaggcctgtacaatgaactgcagaaagataagatggcggaggcctacagtgagattgggatgaaaggcgagcgccggaggggcaaggggcacgatggcctttaccagggtctcagtacagccaccaaggacacctacgacgcccttcacatgcaggccctgccccctcgc